European Patent Specification EP 3 626 074 B1, published March 29, 2023. Title: A transgenic invertebrate animal model for alzheimer's disease, and use thereof. Applicant: National Center for Geriatrics and Gerontology. The sequence listing filed with the application follows.

SEQUENCE LISTING (8 sequences)

SEQ ID NO: 1 - DNA, 20 bp, Artificial Sequence
  GALT6 forward primer
atgtctgtgctcaggcggat

SEQ ID NO: 2 - DNA, 20 bp, Artificial Sequence
  GALT6 reverse primer
cttgccacgacagccacttc

SEQ ID NO: 3 - DNA, 20 bp, Artificial Sequence
  SAT1 forward primer
cattagtatgcggacgaagg

SEQ ID NO: 4 - DNA, 20 bp, Artificial Sequence
  SAT1 reverse primer
gctctcagagttagagttgc

SEQ ID NO: 5 - DNA, 25 bp, Artificial Sequence
  GNE forward primer
catggagaagaatggaaataaccga

SEQ ID NO: 6 - DNA, 20 bp, Artificial Sequence
  GNE reverse primer
ctagtagatcctgcgtgttg

SEQ ID NO: 7 - DNA, 28 bp, Artificial Sequence
  Dut40 forward primer
gtgttctttgcacaagatgtgggttcaa

SEQ ID NO: 8 - DNA, 28 bp, Artificial Sequence
  Dut40 reverse primer
ttgaacccacatcttgtgcaaagaacac